European Patent Application EP 4 245 321 A1, published September 20, 2023. Title: Combination of antibody drug conjugates and anti-SIRP alpha antibodies. Applicant: DAIICHI SANKYO COMPANY, LTD. The sequence listing filed with the application follows.

SEQUENCE LISTING (33 sequences)

SEQ ID NO: 1 - protein, 450 aa, Artificial
  Amino acid sequence of anti HER2 antibody heavy chain
EVQLVESGGGLVQPGGSLRLSCAASGFNIKDTYIHWVRQAPGKGLEWVARIYPTNGYTRYADSVKGRFTISADTSKNTAYLQMNSLRAEDTAVYYCSRWGGDGFYAMDYWGQGTLVTVSSASTKGPSVFPLAPSSKSTSGGTAALGCLVKDYFPEPVTVSWNSGALTSGVHTFPAVLQSSGLYSLSSVVTVPSSSLGTQTYICNVNHKPSNTKVDKKVEPKSCDKTHTCPPCPAPELLGGPSVFLFPPKPKDTLMISRTPEVTCVVVDVSHEDPEVKFNWYVDGVEVHNAKTKPREEQYNSTYRVVSVLTVLHQDWLNGKEYKCKVSNKALPAPIEKTISKAKGQPREPQVYTLPPSREEMTKNQVSLTCLVKGFYPSDIAVEWESNGQPENNYKTTPPVLDSDGSFFLYSKLTVDKSRWQQGNVFSCSVMHEALHNHYTQKSLSLSPGK

SEQ ID NO: 2 - protein, 214 aa, Artificial
  Amino acid sequence of anti HER2 antibody light chain
DIQMTQSPSSLSASVGDRVTITCRASQDVNTAVAWYQQKPGKAPKLLIYSASFLYSGVPSRFSGSRSGTDFTLTISSLQPEDFATYYCQQHYTTPPTFGQGTKVEIKRTVAAPSVFIFPPSDEQLKSGTASVVCLLNNFYPREAKVQWKVDNALQSGNSQESVTEQDSKDSTYSLSSTLTLSKADYEKHKVYACEVTHQGLSSPVTKSFNRGEC

SEQ ID NO: 3 - protein, 447 aa, Homo sapiens
QVQLQQWGAGLLKPSETLSLTCAVYGGSFSGYYWSWIRQPPGKGLEWIGEINHSGSTNYNPSLKSRVTISVETSKNQFSLKLSSVTAADTAVYYCARDKWTWYFDLWGRGTLVTVSSASTKGPSVFPLAPSSKSTSGGTAALGCLVKDYFPEPVTVSWNSGALTSGVHTFPAVLQSSGLYSLSSVVTVPSSSLGTQTYICNVNHKPSNTKVDKRVEPKSCDKTHTCPPCPAPELLGGPSVFLFPPKPKDTLMISRTPEVTCVVVDVSHEDPEVKFNWYVDGVEVHNAKTKPREEQYNSTYRVVSVLTVLHQDWLNGKEYKCKVSNKALPAPIEKTISKAKGQPREPQVYTLPPSREEMTKNQVSLTCLVKGFYPSDIAVEWESNGQPENNYKTTPPVLDSDGSFFLYSKLTVDKSRWQQGNVFSCSVMHEALHNHYTQKSLSLSPGK

SEQ ID NO: 4 - protein, 220 aa, Homo sapiens
DIEMTQSPDSLAVSLGERATINCRSSQSVLYSSSNRNYLAWYQQNPGQPPKLLIYWASTRESGVPDRFSGSGSGTDFTLTISSLQAEDVAVYYCQQYYSTPRTFGQGTKVEIKRTVAAPSVFIFPPSDEQLKSGTASVVCLLNNFYPREAKVQWKVDNALQSGNSQESVTEQDSKDSTYSLSSTLTLSKADYEKHKVYACEVTHQGLSSPVTKSFNRGEC

SEQ ID NO: 5 - protein, 470 aa, Artificial
  Amino acid sequence of anti TROP2 antibody heavy chain
MKHLWFFLLLVAAPRWVLSQVQLVQSGAEVKKPGASVKVSCKASGYTFTTAGMQWVRQAPGQGLEWMGWINTHSGVPKYAEDFKGRVTISADTSTSTAYLQLSSLKSEDTAVYYCARSGFGSSYWYFDVWGQGTLVTVSSASTKGPSVFPLAPSSKSTSGGTAALGCLVKDYFPEPVTVSWNSGALTSGVHTFPAVLQSSGLYSLSSVVTVPSSSLGTQTYICNVNHKPSNTKVDKRVEPKSCDKTHTCPPCPAPELLGGPSVFLFPPKPKDTLMISRTPEVTCVVVDVSHEDPEVKFNWYVDGVEVHNAKTKPREEQYNSTYRVVSVLTVLHQDWLNGKEYKCKVSNKALPAPIEKTISKAKGQPREPQVYTLPPSREEMTKNQVSLTCLVKGFYPSDIAVEWESNGQPENNYKTTPPVLDSDGSFFLYSKLTVDKSRWQQGNVFSCSVMHEALHNHYTQKSLSLSPGK

SEQ ID NO: 6 - protein, 234 aa, Artificial
  Amino acid sequence of anti TROP2 antibody light chain
MVLQTQVFISLLLWISGAYGDIQMTQSPSSLSASVGDRVTITCKASQDVSTAVAWYQQKPGKAPKLLIYSASYRYTGVPSRFSGSGSGTDFTLTISSLQPEDFAVYYCQQHYITPLTFGQGTKLEIKRTVAAPSVFIFPPSDEQLKSGTASVVCLLNNFYPREAKVQWKVDNALQSGNSQESVTEQDSKDSTYSLSSTLTLSKADYEKHKVYACEVTHQGLSSPVTKSFNRGEC

SEQ ID NO: 7 - protein, 471 aa, Artificial
  Amino acid sequence of anti B7-H3 antibody heavy chain
MKHLWFFLLLVAAPRWVLSQVQLVQSGAEVKKPGSSVKVSCKASGYTFTNYVMHWVRQAPGQGLEWMGYINPYNDDVKYNEKFKGRVTITADESTSTAYMELSSLRSEDTAVYYCARWGYYGSPLYYFDYWGQGTLVTVSSASTKGPSVFPLAPSSKSTSGGTAALGCLVKDYFPEPVTVSWNSGALTSGVHTFPAVLQSSGLYSLSSVVTVPSSSLGTQTYICNVNHKPSNTKVDKRVEPKSCDKTHTCPPCPAPELLGGPSVFLFPPKPKDTLMISRTPEVTCVVVDVSHEDPEVKFNWYVDGVEVHNAKTKPREEQYNSTYRVVSVLTVLHQDWLNGKEYKCKVSNKALPAPIEKTISKAKGQPREPQVYTLPPSREEMTKNQVSLTCLVKGFYPSDIAVEWESNGQPENNYKTTPPVLDSDGSFFLYSKLTVDKSRWQQGNVFSCSVMHEALHNHYTQKSLSLSPGK

SEQ ID NO: 8 - protein, 233 aa, Artificial
  Amino acid sequence of anti B7-H3 antibody light chain
MVLQTQVFISLLLWISGAYGEIVLTQSPATLSLSPGERATLSCRASSRLIYMHWYQQKPGQAPRPLIYATSNLASGIPARFSGSGSGTDFTLTISSLEPEDFAVYYCQQWNSNPPTFGQGTKVEIKRTVAAPSVFIFPPSDEQLKSGTASVVCLLNNFYPREAKVQWKVDNALQSGNSQESVTEQDSKDSTYSLSSTLTLSKADYEKHKVYACEVTHQGLSSPVTKSFNRGEC

SEQ ID NO: 9 - protein, 472 aa, Artificial
  Amino acid sequence of anti GPR20 antibody heavy chain
MKHLWFFLLLVAAPRWVLSEVQLVQSGAEVKKPGASVKVSCKASGYTFTSYYISWIRQAPGQGLKYMGFINPGSGHTNYNEKFKGRVTITADKSSSTATMELSSLRSEDTAVYYCARGAGGFLRIITKFDYWGQGTLVTVSSASTKGPSVFPLAPSSKSTSGGTAALGCLVKDYFPEPVTVSWNSGALTSGVHTFPAVLQSSGLYSLSSVVTVPSSSLGTQTYICNVNHKPSNTKVDKRVEPKSCDKTHTCPPCPAPELLGGPSVFLFPPKPKDTLMISRTPEVTCVVVDVSHEDPEVKFNWYVDGVEVHNAKTKPREEQYNSTYRVVSVLTVLHQDWLNGKEYKCKVSNKALPAPIEKTISKAKGQPREPQVYTLPPSREEMTKNQVSLTCLVKGFYPSDIAVEWESNGQPENNYKTTPPVLDSDGSFFLYSKLTVDKSRWQQGNVFSCSVMHEALHNHYTQKSLSLSPGK

SEQ ID NO: 10 - protein, 234 aa, Artificial
  Amino acid sequence of anti GPR20 antibody light chain
MVLQTQVFISLLLWISGAYGDTQLTQSPSSLSASVGDRVTITCRASKSVSTYIHWYQQKPGKQPKLLIYSAGNLESGVPSRFSGSGSGTDFTLTISSLQPEDFANYYCQQINELPYTFGQGTKVEIKRTVAAPSVFIFPPSDEQLKSGTASVVCLLNNFYPREAKVQWKVDNALQSGNSQESVTEQDSKDSTYSLSSTLTLSKADYEKHKVYACEVTHQGLSSPVTKSFNRGEC

SEQ ID NO: 11 - protein, 471 aa, Artificial
  Amino acid sequence of anti CDH6 antibody heavy chain
MKHLWFFLLLVAAPRWVLSEVQLVQSGAEVKKPGASVKVSCKASGYTFTRNFMHWVRQAPGQGLEWMGWIYPGDGETEYAQKFQGRVTITADTSTSTAYMELSSLRSEDTAVYYCARGVYGGFAGGYFDFWGQGTLVTVSSASTKGPSVFPLAPSSKSTSGGTAALGCLVKDYFPEPVTVSWNSGALTSGVHTFPAVLQSSGLYSLSSVVTVPSSSLGTQTYICNVNHKPSNTKVDKRVEPKSCDKTHTCPPCPAPELLGGPSVFLFPPKPKDTLMISRTPEVTCVVVDVSHEDPEVKFNWYVDGVEVHNAKTKPREEQYNSTYRVVSVLTVLHQDWLNGKEYKCKVSNKALPAPIEKTISKAKGQPREPQVYTLPPSREEMTKNQVSLTCLVKGFYPSDIAVEWESNGQPENNYKTTPPVLDSDGSFFLYSKLTVDKSRWQQGNVFSCSVMHEALHNHYTQKSLSLSPGK

SEQ ID NO: 12 - protein, 233 aa, Artificial
  Amino acid sequence of anti CDH6 antibody light chain
MVLQTQVFISLLLWISGAYGDIQMTQSPSSLSASVGDRVTITCKASQNIYKNLAWYQQKPGKAPKLLIYDANTLQTGVPSRFSGSGSGSDFTLTISSLQPEDFATYFCQQYYSGWAFGQGTKVEIKRTVAAPSVFIFPPSDEQLKSGTASVVCLLNNFYPREAKVQWKVDNALQSGNSQESVTEQDSKDSTYSLSSTLTLSKADYEKHKVYACEVTHQGLSSPVTKSFNRGEC

SEQ ID NO: 13 - protein, 466 aa, Artificial
  Amino acid sequence of hH1 heavy chain of humanized anti-SIRP alpha antibody hD13
MKHLWFFLLLVAAPRWVLSQVQLVESGGGVVQPGRSLRLSCAASGFTFSDYGMIWVRQAPGKGLEWVASISSSSSYIYYADSVKGRFTISRDNSKNRLYLQMNSLRAEDTAVYYCARRYYGFNYPFDYWGQGTMVTVSSASTKGPSVFPLAPCSRSTSESTAALGCLVKDYFPEPVTVSWNSGALTSGVHTFPAVLQSSGLYSLSSVVTVPSSSLGTKTYTCNVDHKPSNTKVDKRVESKYGPPCPPCPAPEAAGGPSVFLFPPKPKDTLMISRTPEVTCVVVDVSQEDPEVQFNWYVDGVEVHNAKTKPREEQFNSTYRVVSVLTVLHQDWLNGKEYKCKVSNKGLPSSIEKTISKAKGQPREPQVYTLPPSQEEMTKNQVSLTCLVKGFYPSDIAVEWESNGQPENNYKTTPPVLDSDGSFFLYSRLTVDKSRWQEGNVFSCSVMHEALHNHYTQKSLSLSLGK

SEQ ID NO: 14 - protein, 466 aa, Artificial
  Amino acid sequence of hH2 heavy chain of humanized anti-SIRP alpha antibody hD13
MKHLWFFLLLVAAPRWVLSEVQLVESGGGVVQPGRSLRLSCAASGFTFSDYGMIWVRQAPGKGLEWVASISSSSSYIYYADSVKGRFTISRDNSKNTLYLQMNSLRAEDTAVYYCARRYYGFNYPFDYWGQGTMVTVSSASTKGPSVFPLAPCSRSTSESTAALGCLVKDYFPEPVTVSWNSGALTSGVHTFPAVLQSSGLYSLSSVVTVPSSSLGTKTYTCNVDHKPSNTKVDKRVESKYGPPCPPCPAPEAAGGPSVFLFPPKPKDTLMISRTPEVTCVVVDVSQEDPEVQFNWYVDGVEVHNAKTKPREEQFNSTYRVVSVLTVLHQDWLNGKEYKCKVSNKGLPSSIEKTISKAKGQPREPQVYTLPPSQEEMTKNQVSLTCLVKGFYPSDIAVEWESNGQPENNYKTTPPVLDSDGSFFLYSRLTVDKSRWQEGNVFSCSVMHEALHNHYTQKSLSLSLGK

SEQ ID NO: 15 - protein, 234 aa, Artificial
  Amino acid sequence of hL2 light chain of humanized anti-SIRP alpha antibody hD13
MVLQTQVFISLLLWISGAYGAIQLTQSPSSLSASVGQRVTITCGASKSVRTYMHWYQQKPGKAPKLLIYSASNLEAGVPSRFSGSGSGTDFTLTISSLQPEDFATYYCQQSNEPPYTFGQGTKLEIKRTVAAPSVFIFPPSDEQLKSGTASVVCLLNNFYPREAKVQWKVDNALQSGNSQESVTEQDSKDSTYSLSSTLTLSKADYEKHKVYACEVTHQGLSSPVTKSFNRGEC

SEQ ID NO: 16 - protein, 234 aa, Artificial
  Amino acid sequence of hL3 light chain of humanized anti-SIRP alpha antibody hD13
MVLQTQVFISLLLWISGAYGDTQLTQSPSSLSASVGQRVTITCGASKSVRTYMHWYQQKPGKQPKLLIYSASNLEAGVPSRFSGSGSGTDFTLTISSLQPEDFATYYCQQSNEPPYTFGQGTKLEIKRTVAAPSVFIFPPSDEQLKSGTASVVCLLNNFYPREAKVQWKVDNALQSGNSQESVTEQDSKDSTYSLSSTLTLSKADYEKHKVYACEVTHQGLSSPVTKSFNRGEC

SEQ ID NO: 17 - protein, 234 aa, Artificial
  Amino acid sequence of hL4 light chain of humanized anti-SIRP alpha antibody hD13
MVLQTQVFISLLLWISGAYGDTVLTQSPDSLAVSLGQRATINCGASKSVRTYMHWYQQKPGQQPKLLIYSASNLEAGVPSRFSGSGSGTDFTLTISSLQAEDVAVYYCQQSNEPPYTFGQGTKVEIKRTVAAPSVFIFPPSDEQLKSGTASVVCLLNNFYPREAKVQWKVDNALQSGNSQESVTEQDSKDSTYSLSSTLTLSKADYEKHKVYACEVTHQGLSSPVTKSFNRGEC

SEQ ID NO: 18 - protein, 10 aa, Artificial
  Amino acid sequence of CDR-H1 of chimeric SIRP alpha antibody cD13
GFTFSDYGMI

SEQ ID NO: 19 - protein, 10 aa, Artificial
  Amino acid sequence of CDR-H2 of chimeric SIRP alpha antibody cD13
SISSSSSYIY

SEQ ID NO: 20 - protein, 11 aa, Artificial
  Amino acid sequence of CDR-H3 of chimeric SIRP alpha antibody cD13
RYYGFNYPFDY

SEQ ID NO: 21 - protein, 11 aa, Artificial
  Amino acid sequence of CDR-L1 of chimeric SIRP alpha antibody cD13
GASKSVRTYMH

SEQ ID NO: 22 - protein, 7 aa, Artificial
  Amino acid sequence of CDR-L2 of chimeric SIRP alpha antibody cD13
SASNLEA

SEQ ID NO: 23 - protein, 9 aa, Artificial
  Amino acid sequence of CDR-L3 of chimeric SIRP alpha antibody cD13
QQSNEPPYT

SEQ ID NO: 24 - protein, 466 aa, Artificial
  Amino acid sequence of OSE-172 antibody heavy chain (OSE-172-hG4Pro)
MKHLWFFLLLVAAPRWVLSEVQLVQSGAEVKKPGESLRISCKASGYSFTSYWVHWVRQMPGKGLEWMGNIDPSDSDTHYSPSFQGHVTLSVDKSISTAYLQLSSLKASDTAMYYCVRGGTGTLAYFAYWGQGTLVTVSSASTKGPSVFPLAPCSRSTSESTAALGCLVKDYFPEPVTVSWNSGALTSGVHTFPAVLQSSGLYSLSSVVTVPSSSLGTKTYTCNVDHKPSNTKVDKRVESKYGPPCPPCPAPEFLGGPSVFLFPPKPKDTLMISRTPEVTCVVVDVSQEDPEVQFNWYVDGVEVHNAKTKPREEQFNSTYRVVSVLTVLHQDWLNGKEYKCKVSNKGLPSSIEKTISKAKGQPREPQVYTLPPSQEEMTKNQVSLTCLVKGFYPSDIAVEWESNGQPENNYKTTPPVLDSDGSFFLYSRLTVDKSRWQEGNVFSCSVMHEALHNHYTQKSLSLSPGK

SEQ ID NO: 25 - protein, 239 aa, Artificial
  Amino acid sequence of OSE-172 antibody light chain (OSE-172-hK)
MVLQTQVFISLLLWISGAYGDVVMTQSPLSLPVTLGQPASISCRSSQSLVHSYGNTYLYWFQQRPGQSPRLLIYRVSNRFSGVPDRFSGSGSGTDFTLKISRVEAEDVGVYYCFQGTHVPYTFGGGTKVEIKRTVAAPSVFIFPPSDEQLKSGTASVVCLLNNFYPREAKVQWKVDNALQSGNSQESVTEQDSKDSTYSLSSTLTLSKADYEKHKVYACEVTHQGLSSPVTKSFNRGEC

SEQ ID NO: 26 - protein, 459 aa, Artificial
  Amino acid sequence of KWAR23 antibody heavy chain (KWAR23_hG4Pro)
MKHLWFFLLLVAAPRWVLSEVQLQQSGAELVKPGASVKLSCTASGFNIKDYYIHWVQQRTEQGLEWIGRIDPEDGETKYAPKFQDKATITADTSSNTAYLHLSSLTSEDTAVYYCARWGAYWGQGTLVTVSAASTKGPSVFPLAPCSRSTSESTAALGCLVKDYFPEPVTVSWNSGALTSGVHTFPAVLQSSGLYSLSSVVTVPSSSLGTKTYTCNVDHKPSNTKVDKRVESKYGPPCPPCPAPEFLGGPSVFLFPPKPKDTLMISRTPEVTCVVVDVSQEDPEVQFNWYVDGVEVHNAKTKPREEQFNSTYRVVSVLTVLHQDWLNGKEYKCKVSNKGLPSSIEKTISKAKGQPREPQVYTLPPSQEEMTKNQVSLTCLVKGFYPSDIAVEWESNGQPENNYKTTPPVLDSDGSFFLYSRLTVDKSRWQEGNVFSCSVMHEALHNHYTQKSLSLSLGK

SEQ ID NO: 27 - protein, 235 aa, Artificial
  Amino acid sequence of KWAR23 antibody light chain (KWAR23_hK)
MVLQTQVFISLLLWISGAYGQIVLTQSPAIMSASPGEKVTLTCSASSSVSSSYLYWYQQKPGSSPKLWIYSTSNLASGVPARFSGSGSGTSYSLTISSMEAEDAASYFCHQWSSYPRTFGAGTKLELKRTVAAPSVFIFPPSDEQLKSGTASVVCLLNNFYPREAKVQWKVDNALQSGNSQESVTEQDSKDSTYSLSSTLTLSKADYEKHKVYACEVTHQGLSSPVTKSFNRGEC

SEQ ID NO: 28 - protein, 467 aa, Artificial
  Amino acid sequence of ADU-1805 antibody heavy chain (ADU-1805-hG2)
MKHLWFFLLLVAAPRWVLSEVQLVQSGAEVVKPGASVKLSCKASGSTFTSYWMHWVKQAPGQGLEWIGAIYPVNSDTTYNQKFKGKATLTVDKSASTAYMELSSLRSEDTAVYYCTRSFYYSLDAAWFVYWGQGTLVTVSSASTKGPSVFPLAPCSRSTSESTAALGCLVKDYFPEPVTVSWNSGALTSGVHTFPAVLQSSGLYSLSSVVTVPSSNFGTQTYTCNVDHKPSNTKVDKTVERKCCVECPPCPAPPVAGPSVFLFPPKPKDTLMISRTPEVTCVVVDVSHEDPEVQFNWYVDGVEVHNAKTKPREEQFNSTFRVVSVLTVVHQDWLNGKEYKCKVSNKGLPAPIEKTISKTKGQPREPQVYTLPPSREEMTKNQVSLTCLVKGFYPSDIAVEWESNGQPENNYKTTPPMLDSDGSFFLYSKLTVDKSRWQQGNVFSCSVMHEALHNHYTQKSLSLSPGK

SEQ ID NO: 29 - protein, 234 aa, Artificial
  Amino acid sequence of ADU-1805 antibody light chain (ADU-1805-hK)
MVLQTQVFISLLLWISGAYGDIQMTQSPSSLSASVGDRVTITCRASQDIGSRLNWLQQKPGKAPKRLIYATSSLDSGVPSRFSGSGSGTEFTLTISSLQPEDFATYYCLQYASSPFTFGGGTKVEIKRTVAAPSVFIFPPSDEQLKSGTASVVCLLNNFYPREAKVQWKVDNALQSGNSQESVTEQDSKDSTYSLSSTLTLSKADYEKHKVYACEVTHQGLSSPVTKSFNRGEC

SEQ ID NO: 30 - protein, 460 aa, Mus musculus
MKHLWFFLLLVAAPRWVLSEVQLVESGGGLVQPGGSLKLSCAASGFTFSNYDMAWVRQAPTKGLEWVASISTRGGSSYYRDSVKGRFTVSRDNAKSTLYLQMDSLRSEDTATYYCARHPGDYFDYWGQGVMVTVSSAKTTPPSVYPLAPGSAAQTNSMVTLGCLVKGYFPEPVTVTWNSGSLSSGVHTFPAVLQSDLYTLSSSVTVPSSTWPSETVTCNVAHPASSTKVDKKIVPRDCGCKPCICTVPEVSSVFIFPPKPKDVLTITLTPKVTCVVVAISKDDPEVQFSWFVDDVEVHTAQTQPREEQFNSTFRSVSELPIMHQDWLNGKEFKCRVNSAAFPAPIEKTISKTKGRPKAPQVYTIPPPKEQMAKDKVSLTCMITDFFPEDITVEWQWNGQPAENYKNTQPIMDTDGSYFVYSKLNVQKSNWEAGNTFTCSVLHEGLHNHHTEKSLSHSPGK

SEQ ID NO: 31 - protein, 233 aa, Mus musculus
MVLQTQVFISLLLWISGAYGDTVLTQSPALAVSPGERVTISCRASESVSTLIHWYQQKPGQQPKLLIYLTSHLESGVPARFSGSGSGTDFTLTIDPVEADDTATYYCQQSWTHPWTFGGGTKLELKRADAAPTVSIFPPSSEQLTSGGASVVCFLNNFYPKDINVKWKIDGSERQNGVLNSWTDQDSKDSTYSMSSTLTLTKDEYERHNSYTCEATHKTSTSPIVKSFNRNEC

SEQ ID NO: 32 - protein, 461 aa, Mus musculus
MKHLWFFLLLVAAPRWVLSEVQLVESGGGLVQPGGSLRLSCAASGFTFSDSWIHWVRQAPGKGLEWVAWISPYGGSTYYADSVKGRFTISADTSKNTAYLQMNSLRAEDTAVYYCARRHWPGGFDYWGQGTLVTVSAAKTTPPSVYPLAPGSAAQTNSMVTLGCLVKGYFPEPVTVTWNSGSLSSGVHTFPAVLQSDLYTLSSSVTVPSSTWPSETVTCNVAHPASSTKVDKKIVPRDCGCKPCICTVPEVSSVFIFPPKPKDVLTITLTPKVTCVVVDISKDDPEVQFSWFVDDVEVHTAQTQPREEQFNSTFRSVSELPIMHQDWLNGKEFKCRVNSAAFPAPIEKTISKTKGRPKAPQVYTIPPPKEQMAKDKVSLTCMITDFFPEDITVEWQWNGQPAENYKNTQPIMDTDGSYFVYSKLNVQKSNWEAGNTFTCSVLHEGLHNHHTEKSLSHSPGK

SEQ ID NO: 33 - protein, 234 aa, Mus musculus
MVLQTQVFISLLLWISGAYGDIQMTQSPSSLSASVGDRVTITCRASQDVSTAVAWYQQKPGKAPKLLIYSASFLYSGVPSRFSGSGSGTDFTLTISSLQPEDFATYYCQQYLYHPATFGQGTKVEIKRADAAPTVSIFPPSSEQLTSGGASVVCFLNNFYPKDINVKWKIDGSERQNGVLNSWTDQDSKDSTYSMSSTLTLTKDEYERHNSYTCEATHKTSTSPIVKSFNRNEC